European Patent Application EP 4 736 888 A1, published May 6, 2026. Title: Composition for preventing, improving, or treating the mitochondrial complex 1 associated diseases comprising recombinant adeno-associated virus vector loading Hydra NDi1. Applicant: SAMSUNG LIFE PUBLIC WELFARE FOUNDATION. Application KR. The sequence listing filed with the application follows.

SEQUENCE LISTING (1 sequence)

SEQ ID NO: 1 - DNA, 1365 bp, synthetic construct
  source 1..1365: mol_type = other DNA
agttttagaatttataccagcagctagttataagcgcaaaatgccattctctttatcatctgttctgtatcggaaaagacttgttttattaggaacaggatggggatgttatagtgtgttaaaaaatattaacaagaagctttatgatgtgattgttgttagtccacgaaatcattttctttttacacccttgttaaatagcacaactgttgggactttagaatttcgaagcataattgaaccgattcgaaacactaagtttcgggatgatcatcattttcaattggctgaagcaattcacttaaatccacatgataaattagttgtttgtaaagcagtctcatctgataaagaatatactttatcatacgataaagttgtaattggtgttggagctgttagtaatacttttggaattcctggtgtcccaaagtatgcatattttttgaaagaaatagcagatgctagaaaaatacgtaatcaaatcatatctaattttgagcaaagtttgtttccatatgtaaatgaagaggaaaggttatcactgttgcattttgtcattgttggtggtggtccaactggtattgaatttggagctgagttgtatgactttataacacatgatgttgcaagactttttccaggagagaagaatgatgttcatgtaacattagttgaaggagattcaatattaccttcatttgaccagcgattacgtaaatttgctgagagaaaaattacacaaagagaaaatttccacttaatcaaagattttgttgtggaagttggtgaaaactatgtgaagttgaaatcaggaaaagttcttttaactaagcttgtagtgtggtcaaccggtcttggtcccagaaagtttatagaaagtttagacctacctaaaggtaaatcaaaacaactcaaggtagatgatcatcttcgtgtagttggttatgacagtatatttgcaattggtgattgttcatacatagatggatctcctttaccaagcacggctcaagtggctgaaagacaaggtcgatatgttgcacagtacttatccttattagaaacaaattctaaaacagacagtaaaccatttatgtggtccaatgctggtatgcttgcatatattggtggatataaagctgttgcagatcttccaacaaaagctgggaagataactggatttaaaagttggttaatatggcgatcggtttatcttactcgcttagggagctggagaaatcgaatgcaagttccatttgactgggctaggacttttttttttggcagggatatatctaggttttaaattacaaactttatttaatatttagtattttttgtatcttattaatttgtttttaa